European Patent Specification EP 3 638 304 B1, published July 31, 2024. Title: ZIKA VIRUS STRAINS FOR TREATMENT OF GLIOBLASTOMA. Applicant: WASHINGTON UNIVERSITY UNIVERSITY OF TEXAS MEDICAL BRANCH CLEVELAND CLINIC LERNER RESEARCH INSTITUTE DIAMOND, Michael CHHEDA, Milan RICH, Jeremy SHI, Pei-Yong ZHU, Zhe GORMAN, Matthew. The sequence listing filed with the application follows.

SEQUENCE LISTING (19 sequences)

SEQ ID NO: 1 - DNA, 28 bp, Artificial Sequence
  SYNTHESIZED/PRIMER 1
ccaccaatgttctcttgcagacatattg

SEQ ID NO: 2 - DNA, 26 bp, Artificial Sequence
  SYNTHESIZED/PRIMER 2
ttcggacagccgttgtccaacacaag

SEQ ID NO: 3 - DNA, 21 bp, Artificial Sequence
  SYNTHESIZED/PRIMER 3
agcctaccttgacaagcagtc

SEQ ID NO: 4 - DNA, 21 bp, Artificial Sequence
  SYNTHESIZED/PRIMER 4
aacaggagcgatgagtctgtc

SEQ ID NO: 5 - DNA, 23 bp, Artificial Sequence
  SYNTHESIZED/PRIMER 5
tgcgaaatggtgtaaatgagtca

SEQ ID NO: 6 - DNA, 23 bp, Artificial Sequence
  SYNTHESIZED/PRIMER 6
cagcttgactcaaaattcctgga

SEQ ID NO: 7 - DNA, 23 bp, Artificial Sequence
  SYNTHESIZED/PRIMER 7
tgaagattacgcttgcttttcct

SEQ ID NO: 8 - DNA, 19 bp, Artificial Sequence
  SYNTHESIZED/PRIMER 8
atgcccatcactcggatgc

SEQ ID NO: 9 - DNA, 20 bp, Artificial Sequence
  SYNTHESIZED/PRIMER 9
ccctgctttgtatcggcctg

SEQ ID NO: 10 - DNA, 16 bp, Artificial Sequence
  SYNTHESIZED/PRIMER 10
acgatgaaatgcctga

SEQ ID NO: 11 - DNA, 20 bp, Artificial Sequence
  SYNTHESIZED/PRIMER 11
caggtcaccagactcctcac

SEQ ID NO: 12 - DNA, 22 bp, Artificial Sequence
  SYNTHESIZED/PRIMER 12
ctcagaagctgggttggtttat

SEQ ID NO: 13 - DNA, 21 bp, Artificial Sequence
  SYNTHESIZED/PRIMER 13
accatctcgtcgatcagtgtc

SEQ ID NO: 14 - DNA, 22 bp, Artificial Sequence
  SYNTHESIZED/PRIMER 14
tcgaatgggtattccacagacg

SEQ ID NO: 15 - DNA, 19 bp, Artificial Sequence
  SYNTHESIZED/PRIMER 15
gtggcgactgtcctctgaa

SEQ ID NO: 16 - DNA, 18 bp, Artificial Sequence
  SYNTHESIZED/PRIMER 16
aacccgttgaaccccatt

SEQ ID NO: 17 - DNA, 20 bp, Artificial Sequence
  SYNTHESIZED/PRIMER 17
ccatccaatcggtagtagcg

SEQ ID NO: 18 - DNA, 19 bp, Artificial Sequence
  SYNTHESIZED/PRIMER 18
cctgttcgacagtcagccg

SEQ ID NO: 19 - DNA, 20 bp, Artificial Sequence
  SYNTHESIZED/PRIMER 19
cgaccaaatccgttgactcc